European Patent Specification EP 3 842 050 B1, published June 12, 2024. Title: Recombinant Bifidobacterium expressing antibody introducing apotopsis of cancer cells. Applicant: Teikyo Heisei University. Application Divisional application of EPA 14878071.1. The sequence listing filed with the application follows.

SEQUENCE LISTING (29 sequences)

SEQ ID NO: 1 - DNA, 2064 bp, Artificial
  Synthetic
aagctttgggcgcggcggccatgaagtggcttgacaagcacaatctcgtctgatttttgcccttgccctcccctcgaaaaaaacacataaatcctatataaaatgcgggttttcgcagtcacatgcgctattatcattgattgaacgggcaaagcaacaaatgccgccccctgaccaagaaggatgctttatgaccaatgtgcgcgtcatcaagcctgcactggccgccctggttgccgccgccgcatgcgtgggcgggctggcctttagcagcgcgcagccggcccaggctgacacctatgaagtccagctggtagagagcggaggcggcagcgtacaggccggggacagcctgagactgtcctgcgcggctagtggccgtacctttggctccataagggttgggtggttccgccaaaccccgggcaaggagcgtgagtttgtcgcggccataaaccgcaacgatggtacgacctattatgccgacagcgtcaagggccggttcaccatcagtcgtgacaacgctaagaacactgtttacatgcagatggcatccctgaagcccgaggataccgccgtgtactattgcgcagctgggctgcaatacaaccgcagcgcggaccgcgtgcctgtcggcgcagtatactggggccaaggcacccaagtgacggtgtccagtggcggtagtggcggaggcggctcgggcggagaggtgcagctcgtcgaaagtggcggaggtagcgtgcaggcgggcgattcgctgcgtttgtcgtgcgcggccagcggccggacattcggttccatccgcgtcggttggttccgccagactccgggtaaagaaagggagttcgtggccgccatcaaccgtaacgacggtaccacttactatgccgactccgtgaaagggcgctttacaatctcgcgcgacaacgcgaagaatacggtttacatgcagatggcaagcctcaaaccggaggacacggccgtatactattgcgccgcgggcctgcagtacaaccggtccgccgacagggtgccggtcggggccgtgtactggggtcagggtacccaggtgactgtctccagcggtggaagtggaggtggtggcagcggtggggaggtccagctggtggaatccggcggcggatccgtgcaagcgggagatagtctgcgcttgtcgtgcgcagcgtccggccgcacctttggcagcattcgtgtgggctggttcaggcagaccccaggcaaagagcgggaattcgtggccgctatcaaccgcaatgacggcacaacatattacgccgattccgtcaagggacggttcacgatctcccgcgacaatgcgaagaacaccgtgtatatgcagatggcgtcgcttaaaccggaagataccgccgtctactactgcgctgccggccttcagtataaccgctccgcagaccgtgtcccggtgggcgccgtgtattggggtcaaggcacccaggtcaccgtcagttcgggcggctccggaggaggcggctccggaggcgaagtgcagctggtcgaatccggcggtggttcggtgcaggccggagactccctccgcctgtcctgtgcggcgtccggacgtaccttcggatccattcgcgtcggatggtttcgtcagacaccgggcaaggaaagagagttcgtggcggccattaatcggaatgacggaaccacgtattatgcagactcggttaaggggcgcttcactatcagccgcgataacgccaagaacacggtctacatgcaaatggcctccctcaaacccgaggatacggccgtttattactgtgcggctggcttgcagtataacaggtcggccgacagagtccccgtgggcgctgtctattggggccagggcacccaggtaacggtttcctcccaccaccatcaccaccattgaactagtccttctgctcgtagcgattacttcgagcattactgacgacaaagaccccgaccgagatggtcggggtctttttgttgtggtgctgtgacgtgttgtccaaccgtattattccggactagatcagcggcggccgc

SEQ ID NO: 2 - DNA, 2340 bp, Artificial
  Synthetic
aagctttgggcgcggcggccatgaagtggcttgacaagcacaatctcgtctgatttttgcccttgccctcccctcgaaaaaaacacataaatcctatataaaatgcgggttttcgcagtcacatgcgctattatcattgattgaacgggcaaagcaacaaatgccgccccctgaccaagaaggatgctttatgaccaatgtgcgcgtcatcaagcctgcactggccgccctggttgccgccgccgcatgcgtgggcgggctggcctttagcagcgcgcagccggcccaggctgacacctatgaagtccagctggtggaaagcggaggaggctccgtgcaagctggagacagcctgagactgtcctgtgcagcctccggtaggacctttggctcgattcgcgtcggatggttccgtcagacccctggcaaggaacgtgagttcgttgccgccatcaacaggaacgacggcaccacctattacgcggactccgtcaaaggccgcttcaccatctcgagagacaacgccaagaacacggtctacatgcagatggccagcctgaagccggaggacactgcggtctactattgcgctgccgggttgcagtataaccgcagtgccgatcgtgtgccggtaggggccgtctattggggccagggtacccaggtcaccgtgtcctccggcggcagcggaggcggcgggagcggcggtgaagtccagctcgttgaaagcggtggcggatccgtgcaagcgggcgattccctgcggctttcctgcgcagccagtggccggacgttcggtagcatacgtgtcggctggtttcgccaaactccgggcaaagagcgcgagttcgtagcggcgatcaaccgcaatgacggcactacctactacgcagattcggtgaaagggcgcttcacgatttcccgcgacaatgccaagaatacggtgtatatgcagatggcgtcgctcaagcccgaggatacggccgtgtattactgcgccgctggcctgcagtacaacaggagcgcagaccgggtaccagtgggcgcggtttattggggtcagggcacacaggtgacagtgagttcctctagagagggaggcagcctggctgctctgacagcgcaccaggcctgccatctgcccctggaaacgtttacccggcaccgccagccgcgcgggtgggagcaactggagcagtgcggctacccggtccagaggctggtcgctctgtatctcgcggcccgtttgtcctggaatcaggtggatcaggtaattcggaacgccctggcaagccctgggtcgggaggcgatctgggcgaagccataagggaacagccggaacaggccaggctggcccttactctggcggcggcggagtccgagcgcttcgtccgtcagggcaccgggaacgacgaagctggtgccgcgaatgccgacgtggtttccctcacatgcccggtggcggcaggcgaatgcgccgggccggccgactccggcgacgcgcttctggaacgcaactatcccaccggggccgaattcctgggtgatggcggagatgtttccttctccacccgtggcacgcagaactggacggtcgaacggctgttgcaggcgcaccgccagttggaagagagaggttatgtgttcgttggctaccatgggacgttcctggaagccgcccaatccatcgtgttcggtggcgttcgcgcgcgctcccaggatttggacgccatctggaggggattttatatagcgggtgacccggccttggcctatggatacgcgcaggaccaggagccggatgcgcgtgggcgcatacgtaacggcgccctcctgcgcgtgtatgtgcctaggagtagcttgcctggcttctatcgcacgtccctgacgctggcggccccggaggcagcaggcgaagtcgagcgtctgatcggccatccgctgccactgagactggacgccatcaccggaccggaagaggagggcggcaggctcgagactatccttggctggcctctggctgagcgcactgtcgtgattccatccgcgattcccaccgacccgcgtaacgtgggcggcgatctcgatccgtcgtcgatcccggacaaggaacaggcgatcagcgcgcttcccgactacgctagccagcccggtaaaccgccccgcgaggacctgaagcaccaccaccatcatcattgaactagtccttctgctcgtagcgattacttcgagcattactgacgacaaagaccccgaccgagatggtcggggtctttttgttgtggtgctgtgacgtgttgtccaaccgtattattccggactagatcagcggcggccgc

SEQ ID NO: 3 - DNA, 2001 bp, Artificial
  Synthetic
aagctttgggcgcggcggccatgaagtggcttgacaagcacaatctcgtctgatttttgcccttgccctcccctcgaaaaaaacacataaatcctatataaaatgcgggttttcgcagtcacatgcgctattatcattgattgaacgggcaaagcaacaaatgccgccccctgaccaagaaggatgctttatgaccaatgtgcgcgtcatcaagcctgcactggccgccctggttgccgccgccgcatgcgtgggcgggctggcctttagcagcgcgcagccggcccaggctgacacctatgaagtccagctggtggaaagcggaggaggctccgtgcaagctggagacagcctgagactgtcctgtgcagcctccggtaggacctttggctcgattcgcgtcggatggttccgtcagacccctggcaaggaacgtgagttcgttgccgccatcaacaggaacgacggcaccacctattacgcggactccgtcaaaggccgcttcaccatctcgagagacaacgccaagaacacggtctacatgcagatggccagcctgaagccggaggacactgcggtctactattgcgctgccgggttgcagtataaccgcagtgccgatcgtgtgccggtaggggccgtctattggggccagggtacccaggtcaccgtgtcctccggcggcagcggaggcggcgggagcggcggtgaagtccagctcgttgaaagcggtggcggatccgtgcaagcgggcgattccctgcggctttcctgcgcagccagtggccggacgttcggtagcatacgtgtcggctggtttcgccaaactccgggcaaagagcgcgagttcgtagcggcgatcaaccgcaatgacggcactacctactacgcagattcggtgaaagggcgcttcacgatttcccgcgacaatgccaagaatacggtgtatatgcagatggcgtcgctcaagcccgaggatacggccgtgtattactgcgccgctggcctgcagtacaacaggagcgcagaccgggtaccagtgggcgcggtttattggggtcagggcacacaggtgacagtgagttcctctagaggcggttcgggcggaggtggctccggcggtatggtgtccaagggcgaagagctgttcactggcgtggtgccgatcctggtggagctcgacggggacgtgaatggccacaaattcagcgtgtcgggcgaaggcgaaggcgacgccacctacggcaagctgacgctgaaattcatctgcaccacgggcaaactccccgtcccgtggcccaccctggtcacgactctcacctacggggtccagtgcttctcccgttaccctgaccacatgaagcaacacgacttcttcaagtccgcgatgccggagggctacgtgcaggaacgcacgatcttcttcaaggacgacggcaactacaagacccgggccgaggtcaagttcgagggtgacacccttgtgaatcgcatcgagctgaagggaatcgacttcaaagaggacggaaacattctggggcataagctcgagtacaactacaactcgcacaacgtgtacatcatggctgacaagcagaagaacggcatcaaggtgaacttcaagatccgccataacatcgaggatggctccgtccagctcgcggaccattaccagcagaacaccccgattggcgatggtcccgttctcttgccggacaaccactatctgtcgacgcagtccgcgctgtccaaggatccgaacgagaagcgggaccacatggtgcttctcgagttcgtgaccgcagccggcatcaccctgggaatggacgagctgtacaagcaccaccatcaccaccattgaactagtccttctgctcgtagcgattacttcgagcattactgacgacaaagaccccgaccgagatggtcggggtctttttgttgtggtgctgtgacgtgttgtccaaccgtattattccggactagatcagcggcggccgc

SEQ ID NO: 4 - DNA, 1204 bp, Artificial
  Synthetic
ggtacccaacatgaagttatgcatattactggccgtcgtggcctttgttggcctctcgctcggggcaaccatcaaacttcatgatcaatcaattggcacacagcaatgggaacatagccctttgggagagttgtgtccaccaggatctcatagatcagaacatcctggagcctgtaaccggtgcacagagggtgtgggttacaccaatgcttccaacaatttgtttgcttgcctcccatgtacagcttgtaaatcagatgaagaagagagaagtccctgcaccacgaccaggaacacagcatgtcagtgcaaaccaggaactttccggaatgacaattctgctgagatgtgccggaagtgcagcagagggtgccccagagggatggtcaaggtcaaggattgtacgccctggagtgacatcgagtgtgtccacaaagaatcaggcaatggacataatattgaagggagaatggatccccaacctcaatcccaaccagaatgccggtgtcccaaatgtccagcccctgagctcctgggagggccctcagtcttcatcttccccccgaaacccaaggacgtcctctccatttctgggaggcccgaggtcacgtgcgttgtggtagacgtgggccaggaagaccccgaggttagtttcaactggtacattgatggcgctgaggtgcgaacggccaacacgaagccaaaagaggaacagttcaacagcacgtaccgcgtggtcagcgtcctgcccatccggcaccaggactggctgacggggaaggaattcaagtgcaaggtcaacaacaaagctctcccagcccccatcgagaggaccatctccaaggccaaagggcagacccgggagccgcaggtgtacgccctggccccacaccgggaagagctggccaaggacaccgtgagcgtaacatgcctggtaaaagacttctacccagttgacatcaacattgagtggcagaggaacgggcagccagagtcagagggcacctacgccaccacgccgccacagctggacaacgacgggacctacttcctctacagcaagctctcggtgggaaagaacacgtggcagcggggagaaaccttcacctgtgtggtgatgcacgaggccctgcccaaccactacacccagaaatctatcacccagtcttcgggtaaacatcatcaccatcaccattgactcgag

SEQ ID NO: 5 - DNA, 1198 bp, Artificial
  Synthetic
ggtacccaacatgaagttatgcatattactggccgtcgtggcctttgttggcctctcgctcggggctctgatcacccaacaagacctagctccccagcagagagcggccccacaacaaaagaggtccagcccctcagagggattgtgtccacctggacaccatatctcagaagacggtagagattgcatctcctgcaaatatggacaggactatagcactcactggaatgacctccttttctgcttgcgctgcaccaggtgtgattcaggtgaagtggagctaagtccctgcaccacgaccagaaacacagtgtgtcagtgcgaagaaggcaccttccgggaagaagattctcctgagatgtgccggaagtgccgcacagggtgtcccagagggatggtcaaggtcggtgattgtacaccctggagtgacatcgaatgtgtccacaaagaaattgaagggagaatggatccccaacctcaatcccaaccagaatgccggtgtcccaaatgtccagcccctgagctcctgggagggccctcagtcttcatcttccccccgaaacccaaggacgtcctctccatttctgggaggcccgaggtcacgtgcgttgtggtagacgtgggccaggaagaccccgaggttagtttcaactggtacattgatggcgctgaggtgcgaacggccaacacgaagccaaaagaggaacagttcaacagcacgtaccgcgtggtcagcgtcctgcccatccggcaccaggactggctgacggggaaggaattcaagtgcaaggtcaacaacaaagctctcccagcccccatcgagaggaccatctccaaggccaaagggcagacccgggagccgcaggtgtacgccctggccccacaccgggaagagctggccaaggacaccgtgagcgtaacatgcctggtaaaagacttctacccagttgacatcaacattgagtggcagaggaacgggcagccagagtcagagggcacctacgccaccacgccgccacagctggacaacgacgggacctacttcctctacagcaagctctcggtgggaaagaacacgtggcagcggggagaaaccttcacctgtgtggtgatgcacgaggccctgcccaaccactacacccagaaatctatcacccagtcttcgggtaaacatcatcaccatcaccattgactcgag

SEQ ID NO: 6 - DNA, 1189 bp, Artificial
  Synthetic
ggtacccaacatgaagttatgcatattactggccgtcgtggcctttgttggcctctcgctcggggctaacccagcccataatcgtccagctggcctacagcggccggaggagagcccatcaagaggaccctgtctagcaggccagtacctgtcagaagggaactgcaagccttgcagagagggtattgactacaccagccattccaaccattctctggattcatgtattctctgcacagtctgtaaggaagataaagtcgtagaaacccgatgcaacataaccacaaatacggtgtgtcgatgcaaaccaggcacctttgaagataaagactcccctgagatctgccagtcatgctctaactgcactgacggggaagaggaactgacttcctgtacccccagagaaaaccggaagtgtgtctccaaaacggcttgggcatctattgaagggagaatggatccccaacctcaatcccaaccagaatgccggtgtcccaaatgtccagcccctgagctcctgggagggccctcagtcttcatcttccccccgaaacccaaggacgtcctctccatttctgggaggcccgaggtcacgtgcgttgtggtagacgtgggccaggaagaccccgaggttagtttcaactggtacattgatggcgctgaggtgcgaacggccaacacgaagccaaaagaggaacagttcaacagcacgtaccgcgtggtcagcgtcctgcccatccggcaccaggactggctgacggggaaggaattcaagtgcaaggtcaacaacaaagctctcccagcccccatcgagaggaccatctccaaggccaaagggcagacccgggagccgcaggtgtacgccctggccccacaccgggaagagctggccaaggacaccgtgagcgtaacatgcctggtaaaagacttctacccagttgacatcaacattgagtggcagaggaacgggcagccagagtcagagggcacctacgccaccacgccgccacagctggacaacgacgggacctacttcctctacagcaagctctcggtgggaaagaacacgtggcagcggggagaaaccttcacctgtgtggtgatgcacgaggccctgcccaaccactacacccagaaatctatcacccagtcttcgggtaaacatcatcaccatcaccattgactcgag

SEQ ID NO: 7 - DNA, 440 bp, Artificial
  Synthetic
catatggaggtccagttagtagaatccggcggtggctcagtacaagcgggcgattcactgcgcctgagctgtgcggcgtccggccgtacctttggctctatccgcgtaggttggtttcgccagacgccgggcaaagaacgcgaatttgtggctgcgattaaccgcaatgatgggaccacgtactatgcggactccgtcaaaggtcgcttcacgatttctcgcgataacgccaaaaatacggtgtatatgcagatggcatccctgaaaccagaagataccgccgtgtactattgtgcggcaggtctgcagtataatcgctccgccgaccgcgttccagtaggtgccgtctactggggtcagggtacccaggtaaccgttagttcgaagcttgaacaaaaactcatctcagaagaggatctgaatggggccgcagcggccgc

SEQ ID NO: 8 - DNA, 49 bp, Artificial
  Primer
ggtaaaggcccagccggccatggccgaggtgcagctcgtggagtctggg

SEQ ID NO: 9 - DNA, 41 bp, Artificial
  Primer
ttgcaagcaattgcggccgctgaggagacggtgacctgggt

SEQ ID NO: 10 - DNA, 56 bp, Artificial
  Primer
cccatatgtggtcccatccgcagtttgaaaaagacacctatgaagtccagctggta

SEQ ID NO: 11 - DNA, 36 bp, Artificial
  Primer
aattgcggccgctcaatggtggtgatggtggtggga

SEQ ID NO: 12 - DNA, 56 bp, Artificial
  Primer
cccatatgtggtcccatccgcagtttgaaaaagacacctatgaagtccagctggtg

SEQ ID NO: 13 - DNA, 36 bp, Artificial
  Primer
aattgcggccgccttcaggtcctggcggggcggttt

SEQ ID NO: 14 - DNA, 44 bp, Artificial
  Primer
ttgcaagcaattgcggccgccttgtacagctcgtccattcccag

SEQ ID NO: 15 - protein, 5 aa, Artificial
  Recombinant construct
SIRVG

SEQ ID NO: 16 - protein, 17 aa, Artificial
  Recombinant construct
AINRNDGTTYYADSVKG

SEQ ID NO: 17 - protein, 17 aa, Artificial
  Recombinant construct
GLQYNRSADRVPVGAVY

SEQ ID NO: 18 - protein, 30 aa, Artificial
  Recombinant construct
QGIKARSQFVESGGGLVQPGGSLRLSCTAS

SEQ ID NO: 19 - protein, 17 aa, Artificial
  Recombinant construct
VGWFRQAPGKEREGVLC

SEQ ID NO: 20 - protein, 38 aa, Artificial
  Recombinant construct
NVANSVKGRFTISRDNDKNTVYLQMNSLKPEDTSVYYC

SEQ ID NO: 21 - protein, 11 aa, Artificial
  Recombinant construct
WGQGTQVTVSS

SEQ ID NO: 22 - protein, 8 aa, Artificial
  Recombinant construct
GRTFSSNV

SEQ ID NO: 23 - protein, 8 aa, Artificial
  Recombinant construct
IRWRGDST

SEQ ID NO: 24 - protein, 10 aa, Artificial
  Recombinant construct
AASSGNTYLY

SEQ ID NO: 25 - DNA, 184 bp, Artificial
  Synthetic DNA derived from hup promoter of Bifidobacterium longum
tgggcgcggcggccatgaagtggcttgacaagcacaatctcgtctgatttttgcccttgccctcccctcgaaaaaaacacataaatcctatataaaatgcgggttttcgcagtcacatgcgctattatcattgattgaacgggcaaagcaacaaatgccgccccctgaccaagaaggatgcttt

SEQ ID NO: 26 - DNA, 126 bp, Artificial
  Synthetic DNA derived from HUT terminator
ccttctgctcgtagcgattacttcgagcattactgacgacaaagaccccgaccgagatggtcggggtctttttgttgtggtgctgtgacgtgttgtccaaccgtattattccggactagatcagcg

SEQ ID NO: 27 - protein, 6 aa, Artificial
  Synthetic
IEGRMD

SEQ ID NO: 28 - protein, 10 aa, Artificial
  Synthetic
GGSGGGGSGG

SEQ ID NO: 29 - DNA, 102 bp, Artificial
  Synthetic DNA derived from usp secretory signal sequence of Bifidobacterium longum
atgaccaatgtgcgcgtcatcaagcctgcactggccgccctggttgccgccgccgcatgcgtgggcgggctggcctttagcagcgcgcagccggcccaggct